European Patent Application EP 4 653 455 A1, published November 26, 2025. Title: MUTATED PD1 ECTODOMAIN FRAGMENT AND CAR CONTAINING SAME, AND NK CELL. Applicant: Shanghai Metta Therapeutics Co., Ltd. The sequence listing filed with the application follows.

SEQUENCE LISTING (5 sequences)

SEQ ID NO: 1 - protein, 147 aa, synthetic construct
FLDSPDRPWNPPTFSPALLVVTEGDNATFTCSFSNTSESFHVVWHRESPSGQTDTLAAFPEDRSQPGQDCRFRVTQLPNGRDFHMSVVRARRNDSGTYVCGVISLAPKIQIKESLRAELRVTERRAEVPTAHPSPSPRPAGQFQTLV

SEQ ID NO: 2 - DNA, 1203 bp, synthetic construct
  source 1..1203: mol_type = other DNA
gcattgcccgtgaccgccctgctgctgccactggccttgttgctccacgccgcgcggccaatgggatccttcctggactcccctgacagaccctggaaccctcctaccttttcccccgctctgctggtggtgaccgagggagataacgccaccttcacctgcagctttagcaacacctccgagagcttccacgtggtgtggcacagagaatccccctccggacagaccgacaccctggctgctttccctgaagacagaagccagcccggccaggattgcagatttagagtgacccagctgccaaacggcagagattttcacatgagcgtggtgcgcgctagaagaaacgactccggcacctatgtgtgcggcgtgatcagcctggctcccaaaatccagatcaaggaaagcctgagagccgagctgagagtgaccgagagaagagccgaggtgcccacagctcaccctagtcctagccctaggcctgctggacagttccagaccctggtgttcgtgccggtcttcctgccagcgaagcccaccacgacgccagcgccgcgaccaccaacaccggcgcccaccatcgcgtcgcagcccctgtccctgcgcccagaggcgtgccggccagcggcggggggcgcagtgcacacgagggggctggacttcgcctgtgatatctacatctgggcgcccttggccgggacttgtggggtccttctcctgtcactggttatcaccaaacggggcagaaagaaactcctgtatatattcaaacaaccatttatgagaccagtacaaactactcaagaggaagatggctgtagctgccgatttccagaagaagaagaaggaggatgtgaactgagagtgaagttcagcaggagcgcagacgcccccgcgtaccagcagggccagaaccagctctataacgagctcaatctaggacgaagagaggagtacgatgttttggacaagagacgtggccgggaccctgagatggggggaaagccgagaaggaagaaccctcaggaaggcctgtacaatgaactgcagaaagataagatggcggaggcctacagtgagattgggatgaaaggcgagcgccggaggggcaaggggcacgatggcctttaccagggtctcagtacagccaccaaggacacctacgacgcccttcacatgcaggccctgccccctcgctaa

SEQ ID NO: 3 - protein, 400 aa, synthetic construct
ALPVTALLLPLALLLHAARPMGSFLDSPDRPWNPPTFSPALLVVTEGDNATFTCSFSNTSESFHVVWHRESPSGQTDTLAAFPEDRSQPGQDCRFRVTQLPNGRDFHMSVVRARRNDSGTYVCGVISLAPKIQIKESLRAELRVTERRAEVPTAHPSPSPRPAGQFQTLVFVPVFLPAKPTTTPAPRPPTPAPTIASQPLSLRPEACRPAAGGAVHTRGLDFACDIYIWAPLAGTCGVLLLSLVITKRGRKKLLYIFKQPFMRPVQTTQEEDGCSCRFPEEEEGGCELRVKFSRSADAPAYQQGQNQLYNELNLGRREEYDVLDKRRGRDPEMGGKPRRKNPQEGLYNELQKDKMAEAYSEIGMKGERRRGKGHDGLYQGLSTATKDTYDALHMQALPPR

SEQ ID NO: 4 - protein, 147 aa, synthetic construct
FLDSPDRPWNPPTFSPALLVVTEGDNATFTCSFSNTSESFVLNWYRMSPSNQTDKLAAFPEDRSQPGQDCRFRVTQLPNGRDFHMSVVRARRNDSGTYLCGAISLAPKAQIKESLRAELRVTERRAEVPTAHPSPSPRPAGQFQTLV

SEQ ID NO: 5 - protein, 277 aa, synthetic construct
MHSSALLCCLVLLTGVRADSPDRPWNPPTFSPALLVVTEGDNATFTCSFSNTSESFHVVWHRESPSGQTDTLAAFPEDRSQPGQDARFRVTQLPNGRDFHMSVVRARRNDSGTYVCGVISLAPKIQIKESLRAELRVTEREPKSCDKTHTCPPCGGGSSGGGSGGQPREPQVYTLPPSREEMTKNQVSLTCLVKGFYPSDIAVEWESNGQPENNYKTTPPVLDSDGSFFLYSKLTVDKSRWQQGNVFSCSVMHEALHNHYTQKSLSLSPGKHHHHHH